European Patent Specification EP 4 078 181 B1, published March 20, 2024. Title: A method of detecting and/or quantitating an analyte of interest in a plurality of biological liquid samples. Applicant: Blink AG. The sequence listing filed with the application follows.

SEQUENCE LISTING (6 sequences)

SEQ ID NO: 1 - DNA, 20 bp, Artificial Sequence
  "HCV-Brun sense primer"
  HCV-Brun sense primer
gtggtctgcggaaccggtga

SEQ ID NO: 2 - DNA, 22 bp, Artificial Sequence
  "HCV-Brun antisense primer"
  HCV-Brun antisense primer
cgcaagcaccctatcaggcagt

SEQ ID NO: 3 - DNA, 25 bp, Artificial Sequence
  "HCV-Brun TaqMan probe "
  HCV-Brun TaqMan probe
ccgagtagygttgggtygcgaaagg

SEQ ID NO: 4 - DNA, 22 bp, Artificial Sequence
  "MS2-Nino sense Primer"
  MS2-Nino sense Primer
ctctgagagcggctctattggt

SEQ ID NO: 5 - DNA, 24 bp, Artificial Sequence
  "MS2-Nino sense Primer "
  MS2-Nino sense Primer
ggtccctacaacgagcctaaattc

SEQ ID NO: 6 - DNA, 25 bp, Artificial Sequence
  "MS2-Nino TaqMan probe "
  MS2-Nino TaqMan probe
tcagacacgcggtccgctataacga